European Patent Application EP 4 249 499 A1, published September 27, 2023. Title: Therapeutic protein CTP alpha, CTP beta, CTP gamma, CTP delta for treating coronavirus disease COVID-19 and use thereof. Applicant: Daegu Gyeongbuk Institute of Science and Technology. The sequence listing filed with the application follows.

SEQUENCE LISTING (10 sequences)

SEQ ID NO: 1 - protein, 54 aa, Artificial Sequence
  CTP-Alpha1
MKSELASNVYNTNITKENVQNMNEEQAKTFLDKFNHEAEDLFYQSSGLGKGDFR

SEQ ID NO: 2 - protein, 54 aa, Artificial Sequence
  CTP-Alpha2
MKSDLASNVYNTNITKENVQNMNEEQAKTFLDKFNHEAEDLFYQSSGLGKGDFR

SEQ ID NO: 3 - protein, 54 aa, Artificial Sequence
  CTP-Alpha3
MKSQLAENVYNTNITKENVQNMNEEQAKTFLDKFNHEAEDLFYQSSGLGKGDFR

SEQ ID NO: 4 - protein, 54 aa, Artificial Sequence
  CTP-Beta1
MKSELASVNYNTNITKENVQANGEEQAKTFLDKFNHEAEDLFYQSSGLGKGDFR

SEQ ID NO: 5 - protein, 54 aa, Artificial Sequence
  CTP-Beta2
MESELASVNYNTNITKENVQANGEEQAKTFLDKFNHEAEDLFYQSSGLGKGDFR

SEQ ID NO: 6 - protein, 54 aa, Artificial Sequence
  CTP-Beta3
MESELASNVYNTNITKENVQNMNEEQAKTFLDKFNHEAEDLFYQSSGLGKGDFR

SEQ ID NO: 7 - protein, 55 aa, Artificial Sequence
  CTP-Gamma1
MKASSLADNVYNTNITKENVQNMNEEQAKTFLDKFNHEAEDLFYQSSGLGKGDFR

SEQ ID NO: 8 - protein, 55 aa, Artificial Sequence
  CTP-Gamma2
MKESSLADNVYNTNITKENVQNMNEEQAKTFLDKFNHEAEDLFYQSSGLGKGDFR

SEQ ID NO: 9 - protein, 55 aa, Artificial Sequence
  CTP-Gamma3
MKASELADNVYNTNITKENVQNMNEEQAKTFLDKFNHEAEDLFYQSSGLGKGDFR

SEQ ID NO: 10 - protein, 46 aa, Artificial Sequence
  CTP-Delta1
MGEFADKLKNELAKTEEQAKTFLDKFNHEAEDLFYQSSGLGKGDFR